European Patent Application EP 4 233 890 A2, published August 30, 2023. Title: PEPTIDES FOR TREATMENT AND PREVENTION OF DIABETES AND ASSOCIATED DISORDERS. Applicant: UNIVERSITE DE STRASBOURG. Application WO PCT/EP2019/086573, filed December 20, 2019. The sequence listing filed with the application follows.

SEQUENCE LISTING (57 sequences)

SEQ ID NO: 1 - protein, 672 aa, Homo sapiens
MADVFPGNDSTASQDVANRFARKGALRQKNVHEVKDHKFIARFFKQPTFCSHCTDFIWGFGKQGFQCQVCCFVVHKRCHEFVTFSCPGADKGPDTDDPRSKHKFKIHTYGSPTFCDHCGSLLYGLIHQGMKCDTCDMNVHKQCVINVPSLCGMDHTEKRGRIYLKAEVADEKLHVTVRDAKNLIPMDPNGLSDPYVKLKLIPDPKNESKQKTKTIRSTLNPQWNESFTFKLKPSDKDRRLSVEIWDWDRTTRNDFMGSLSFGVSELMKMPASGWYKLLNQEEGEYYNVPIPEGDEEGNMELRQKFEKAKLGPAGNKVISPSEDRKQPSNNLDRVKLTDFNFLMVLGKGSFGKVMLADRKGTEELYAIKILKKDVVIQDDDVECTMVEKRVLALLDKPPFLTQLHSCFQTVDRLYFVMEYVNGGDLMYHIQQVGKFKEPQAVFYAAEISIGLFFLHKRGIIYRDLKLDNVMLDSEGHIKIADFGMCKEHMMDGVTTRTFCGTPDYIAPEIIAYQPYGKSVDWWAYGVLLYEMLAGQPPFDGEDEDELFQSIMEHNVSYPKSLSKEAVSVCKGLMTKHPAKRLGCGPEGERDVREHAFFRRIDWEKLENREIQPPFKPKVCGKGAENFDKFFTRGQPVLTPPDQLVIANIDQSDFEGFSYVNPQFVHPILQSAV

SEQ ID NO: 2 - protein, 257 aa, Homo sapiens
FNFLMVLGKGSFGKVMLADRKGTEELYAIKILKKDVVIQDDDVECTMVEKRVLALLDKPPFLTQLHSCFQTVDRLYFVMEYVNGGDLMYHIQQVGKFKEPQAVFYAAEISIGLFFLHKRGIIYRDLKLDNVMLDSEGHIKIADFGMCKEHMMDGVTTRTFCGTPDYIAPEIIAYQPYGKSVDWWAYGVLLYEMLAGQPPFDGEDEDELFQSIMEHNVSYPKSLSKEAVSVCKGLMTKHPAKRLGCGPEGERDVREHA

SEQ ID NO: 3 - protein, 12 aa, synthetic construct
  REGION 1..12: note = segment of kinase domain of alphaPKC
VECTMVEKRVLA

SEQ ID NO: 4 - protein, 8 aa, synthetic construct
  REGION 1..8: note = segment of kinase domain of alphaPKC
LMYHIQQV

SEQ ID NO: 5 - protein, 4 aa, synthetic construct
  REGION 1..4: note = segment of kinase domain of alphaPKC
PEII

SEQ ID NO: 6 - protein, 16 aa, synthetic construct
  REGION 1..16: note = segment of kinase domain of alphaPKC
SVDWWAYGVLLYEMLA

SEQ ID NO: 7 - protein, 12 aa, synthetic construct
  REGION 1..12: note = segment of kinase domain of alphaPKC
EDEDELFQSIME

SEQ ID NO: 8 - protein, 7 aa, synthetic construct
  REGION 1..7: note = segment of kinase domain of alphaPKC
GERDVRE

SEQ ID NO: 9 - protein, 12 aa, synthetic construct
  REGION 1..12: note = mutated segment of kinase domain of alphaPKC
  SITE 5: note = X is any amino acid except R, M and P
VECTXVEKRVLA

SEQ ID NO: 10 - protein, 12 aa, synthetic construct
  REGION 1..12: note = mutated segment of kinase domain of alphaPKC
  SITE 9: note = X is any amino acid except M, P and R
VECTMVEKXVLA

SEQ ID NO: 11 - protein, 12 aa, synthetic construct
  REGION 1..12: note = mutated segment of kinase domain of alphaPKC
  SITE 5: note = X is any amino acid except M, P and R
  SITE 9: note = X is any amino acid except M, P and R
VECTXVEKXVLA

SEQ ID NO: 12 - protein, 8 aa, synthetic construct
  REGION 1..8: note = mutated segment of kinase domain of alphaPKC
  SITE 2: note = X is any amino acid except M, P and R
LXYHIQQV

SEQ ID NO: 13 - protein, 16 aa, synthetic construct
  REGION 1..16: note = mutated segment of kinase domain of alphaPKC
  SITE 14: note = X is any amino acid except M, P and R
SVDWWAYGVLLYEXLA

SEQ ID NO: 14 - protein, 12 aa, synthetic construct
  REGION 1..12: note = mutated segment of kinase domain of alphaPKC
  SITE 11: note = X is any amino acid except M, P and R
EDEDELFQSIXE

SEQ ID NO: 15 - protein, 7 aa, synthetic construct
  REGION 1..7: note = mutated segment of kinase domain of alphaPKC
  SITE 3: note = X is any amino acid except M, P and R
GEXDVRE

SEQ ID NO: 16 - protein, 7 aa, synthetic construct
  REGION 1..7: note = mutated segment of kinase domain of alphaPKC
  SITE 6: note = X is any amino acid except M, P and R
GERDVXE

SEQ ID NO: 17 - protein, 7 aa, synthetic construct
  REGION 1..7: note = mutated segment of kinase domain of alphaPKC
  SITE 3: note = X is any amino acid except M, P and R
  SITE 6: note = X is any amino acid except M, P and R
GEXDVXE

SEQ ID NO: 18 - skipped

SEQ ID NO: 19 - protein, 12 aa, synthetic construct
  REGION 1..12: note = mutated segment of kinase domain of alphaPKC
VECTTVEKEVLA

SEQ ID NO: 20 - protein, 25 aa, synthetic construct
  REGION 1..25: note = mutated segment of kinase domain of alphaPKC
  SITE 5: note = X is any amino acid except M, P and R
  SITE 9: note = X is any amino acid except M, P and R
  REGION 17..18: note = X is any amino acid except M, P and R
VECTXVEKXVLALLDKXXFLTQLHS

SEQ ID NO: 21 - protein, 25 aa, synthetic construct
  REGION 1..25: note = mutated segment of kinase domain of alphaPKC
  REGION 17..18: note = X is any amino acid except M, P and R
VECTMVEKRVLALLDKXXFLTQLHS

SEQ ID NO: 22 - protein, 25 aa, synthetic construct
  REGION 1..25: note = mutated segment of kinase domain of alphaPKC
  SITE 5: note = X is any amino acid except M, P and R
VECTXVEKRVLALLDKPPFLTQLHS

SEQ ID NO: 23 - protein, 25 aa, synthetic construct
  REGION 1..25: note = mutated segment of kinase domain of alphaPKC
  SITE 9: note = X is any amino acid except M, P and R
VECTMVEKXVLALLDKPPFLTQLHS

SEQ ID NO: 24 - protein, 13 aa, synthetic construct
  REGION 1..13: note = mutated segment of kinase domain of alphaPKC
  SITE 6: note = X is any amino acid derivative suitable for stapling
  SITE 13: note = X is any amino acid derivative suitable for stapling
VECTMXEKRVLAX

SEQ ID NO: 25 - protein, 13 aa, synthetic construct
  REGION 1..13: note = mutated segment of kinase domain of alphaPKC
  SITE 5: note = X is any amino acid except M, P and R
  SITE 6: note = X is any amino acid derivative suitable for stapling
  SITE 13: note = X is any amino acid derivative suitable for stapling
VECTXXEKRVLAX

SEQ ID NO: 26 - protein, 13 aa, synthetic construct
  REGION 1..13: note = mutated segment of kinase domain of alphaPKC
  SITE 6: note = X is any amino acid derivative suitable for stapling
  SITE 9: note = X is any amino acid except M, P and R
  SITE 13: note = X is any amino acid derivative suitable for stapling
VECTMXEKXVLAX

SEQ ID NO: 27 - protein, 13 aa, synthetic construct
  REGION 1..13: note = mutated segment of kinase domain of alphaPKC
  SITE 5: note = X is any amino acid except M, P and R
  SITE 6: note = X is any amino acid derivative suitable for stapling
  SITE 9: note = X is any amino acid except M, P and R
  SITE 13: note = X is any amino acid derivative suitable for stapling
VECTXXEKXVLAX

SEQ ID NO: 28 - protein, 25 aa, synthetic construct
  REGION 1..25: note = mutated segment of kinase domain of alphaPKC
  SITE 5: note = X is any amino acid except M, P and R
  SITE 6: note = X is any amino acid derivative suitable for stapling
  SITE 9: note = X is any amino acid except M, P and R
  SITE 13: note = X is any amino acid derivative suitable for stapling
  REGION 17..18: note = X is any amino acid except M, P and R
VECTXXEKXVLAXLDKXXFLTQLHS

SEQ ID NO: 29 - protein, 25 aa, synthetic construct
  REGION 1..25: note = mutated segment of kinase domain of alphaPKC
  SITE 6: note = X is any amino acid derivative suitable for stapling
  SITE 13: note = X is any amino acid derivative suitable for stapling
  REGION 17..18: note = X is any amino acid except M, P and R
VECTMXEKRVLAXLDKXXFLTQLHS

SEQ ID NO: 30 - protein, 25 aa, synthetic construct
  REGION 1..25: note = mutated segment of kinase domain of alphaPKC
  SITE 5: note = X is any amino acid except M, P and R
  SITE 6: note = X is any amino acid derivative suitable for stapling
  SITE 13: note = X is any amino acid derivative suitable for stapling
VECTXXEKRVLAXLDKPPFLTQLHS

SEQ ID NO: 31 - protein, 25 aa, synthetic construct
  REGION 1..25: note = mutated segment of kinase domain of alphaPKC
  SITE 6: note = X is any amino acid derivative suitable for stapling
  SITE 9: note = X is any amino acid except M, P and R
  SITE 13: note = X is any amino acid derivative suitable for stapling
VECTMXEKXVLAXLDKPPFLTQLHS

SEQ ID NO: 32 - protein, 25 aa, synthetic construct
  REGION 1..25: note = mutated segment of kinase domain of alphaPKC
  SITE 6: note = 2-(7-octenyl)arginine
  SITE 13: note = 2-(4-pentenyl)serine
VECTTREKEVLASLDKAAFLTQLHS

SEQ ID NO: 33 - protein, 8 aa, synthetic construct
  REGION 1..8: note = protein transduction domain
RRRRRRRR

SEQ ID NO: 34 - protein, 15 aa, synthetic construct
  REGION 1..15: note = protein transduction domain
RRPRRPRRPRRPRRP

SEQ ID NO: 35 - protein, 16 aa, synthetic construct
  REGION 1..16: note = penetratin peptide
RQIKIWFQNRRMKWKK

SEQ ID NO: 36 - protein, 11 aa, synthetic construct
  REGION 1..11: note = HIV-tat
YGRKKRRQRRR

SEQ ID NO: 37 - DNA, 20 bp, synthetic construct
  misc_feature 1..20: note = primer
  source 1..20: mol_type = other DNA
tgctttggtttctgggactt

SEQ ID NO: 38 - DNA, 20 bp, synthetic construct
  misc_feature 1..20: note = primer
  source 1..20: mol_type = other DNA
gctctagccgaacacgaatc

SEQ ID NO: 39 - DNA, 22 bp, synthetic construct
  misc_feature 1..22: note = primer
  source 1..22: mol_type = other DNA
tggacaaagtagacggagtgtc

SEQ ID NO: 40 - DNA, 20 bp, synthetic construct
  misc_feature 1..20: note = primer
  source 1..20: mol_type = other DNA
tagcaaggcctgtcccatac

SEQ ID NO: 41 - DNA, 20 bp, synthetic construct
  misc_feature 1..20: note = primer
  source 1..20: mol_type = other DNA
tgagaacttgccaccgtatg

SEQ ID NO: 42 - DNA, 20 bp, synthetic construct
  misc_feature 1..20: note = primer
  source 1..20: mol_type = other DNA
ggcaggtaggcccctatatc

SEQ ID NO: 43 - DNA, 20 bp, synthetic construct
  misc_feature 1..20: note = primer
  source 1..20: mol_type = other DNA
gtttcatccgggtcttcatc

SEQ ID NO: 44 - DNA, 20 bp, synthetic construct
  misc_feature 1..20: note = primer
  source 1..20: mol_type = other DNA
gtgtctgtgccctcgaaaat

SEQ ID NO: 45 - DNA, 20 bp, synthetic construct
  misc_feature 1..20: note = primer
  source 1..20: mol_type = other DNA
aagttctctgcctcccgatt

SEQ ID NO: 46 - DNA, 20 bp, synthetic construct
  misc_feature 1..20: note = primer
  source 1..20: mol_type = other DNA
caaagcgttgctggaagttt

SEQ ID NO: 47 - DNA, 20 bp, synthetic construct
  misc_feature 1..20: note = primer
  source 1..20: mol_type = other DNA
tcgattccctcctacactgc

SEQ ID NO: 48 - DNA, 20 bp, synthetic construct
  misc_feature 1..20: note = primer
  source 1..20: mol_type = other DNA
ttggtggtactggctcatca

SEQ ID NO: 49 - protein, 25 aa, synthetic construct
  REGION 1..25: note = PATAD
  SITE 6: note = 2-(4-pentenyl) alanine
  SITE 13: note = 2-(4-pentenyl)alanine
VECTMAEKRVLAALDKPPFLTQLHS

SEQ ID NO: 50 - protein, 13 aa, synthetic construct
  REGION 1..13: note = segment of kinase domain of alphaPKC
ECTMVEKKVLALL

SEQ ID NO: 51 - protein, 15 aa, synthetic construct
  REGION 1..15: note = mutated segment of kinase domain of alphaPKC
SVEWWAYGLLYEMLA

SEQ ID NO: 52 - protein, 15 aa, synthetic construct
  REGION 1..15: note = mutated segment of kinase domain of alphaPKC
  SITE 3: note = X is any amino acid except M, P and R
SVXWWAYGLLYEMLA

SEQ ID NO: 53 - protein, 24 aa, synthetic construct
  REGION 1..24: note = mutated segment of kinase domain of alphaPKC
  SITE 6: note = X is any amino acid derivative suitable for stapling
  SITE 13: note = X is any amino acid derivative suitable for stapling
VECTTXEKEVLAXLDKAAFLTQHS

SEQ ID NO: 54 - protein, 19 aa, synthetic construct
  REGION 1..19: note = mutated segment of kinase domain of alphaPKC
  SITE 6: note = X is any amino acid derivative suitable for stapling
  SITE 13: note = X is any amino acid derivative suitable for stapling
VECTTXEKEVLAXLDKAAF

SEQ ID NO: 55 - protein, 19 aa, synthetic construct
  REGION 1..19: note = mutated segment of kinase domain of alphaPKC
  SITE 6: note = X is any amino acid derivative suitable for stapling
  SITE 13: note = X is any amino acid derivative suitable for stapling
VEGTTXEKEVLAXLDKAAF

SEQ ID NO: 56 - protein, 13 aa, synthetic construct
  REGION 1..13: note = mutated segment of kinase domain of alphaPKC
  SITE 5: note = X is any amino acid derivative suitable for stapling
  SITE 12: note = X is any amino acid derivative suitable for stapling
ECTTXEKEVLAXL

SEQ ID NO: 57 - protein, 13 aa, synthetic construct
  REGION 1..13: note = mutated segment of kinase domain of alphaPKC
  SITE 5: note = X is any amino acid derivative suitable for stapling
  SITE 12: note = X is any amino acid derivative suitable for stapling
ECTMXEKKVLAXL